European Patent Application EP 4 786 593 A1, published August 5, 2026. Title: 包含多个双链寡核苷酸分子的核酸嵌合体、组合物及其用途. Applicant: 北京炫景瑞医药科技有限公司. The sequence listing filed with the application follows.

SEQUENCE LISTING (11 sequences)

SEQ ID NO: 1 - RNA, 19 nt, artificial sequence
  source 1..19: mol_type = genomic RNA
ttttaatcctcactctaaa

SEQ ID NO: 2 - RNA, 19 nt, artificial sequence
  source 1..19: mol_type = genomic RNA
ccaagagcaccaagaacta

SEQ ID NO: 3 - RNA, 21 nt, artificial sequence
  source 1..21: mol_type = genomic RNA
tttagagtgaggattaaaatg

SEQ ID NO: 4 - RNA, 21 nt, artificial sequence
  source 1..21: mol_type = genomic RNA
tagttcttggtgctcttggtt

SEQ ID NO: 5 - RNA, 20 nt, artificial sequence
  source 1..20: mol_type = genomic RNA
tttagagtgaggattaaaat

SEQ ID NO: 6 - DNA, 19 bp, artificial sequence
  source 1..19: mol_type = genomic DNA
tgcaccaccaactgcttag

SEQ ID NO: 7 - DNA, 19 bp, artificial sequence
  source 1..19: mol_type = genomic DNA
ggatgcagggatgatgttc

SEQ ID NO: 8 - DNA, 23 bp, artificial sequence
  source 1..23: mol_type = genomic DNA
gaggagcagctaaccaacttaat

SEQ ID NO: 9 - DNA, 23 bp, artificial sequence
  source 1..23: mol_type = genomic DNA
tctgcatgtgctgttgacttaat

SEQ ID NO: 10 - DNA, 20 bp, artificial sequence
  source 1..20: mol_type = genomic DNA
gggttccacgtccatcagta

SEQ ID NO: 11 - DNA, 20 bp, artificial sequence
  source 1..20: mol_type = genomic DNA
acaccgtcctttccagcagt